European Patent Specification EP 3 061 828 B1, published August 28, 2024. Title: Method for producing target substance. Applicant: Ajinomoto Co., Inc. The sequence listing filed with the application follows.

SEQUENCE LISTING (47 sequences)

SEQ ID NO: 1 - DNA, 35 bp, Artificial Sequence
  primer
ccaggaggacatacaatgcaagcctattttgacca

SEQ ID NO: 2 - DNA, 35 bp, Artificial Sequence
  primer
gcaggtcgactctagttacgccattaatggcagaa

SEQ ID NO: 3 - DNA, 35 bp, Artificial Sequence
  primer
ccggggatcctctagagatcgtttagatccgaagg

SEQ ID NO: 4 - DNA, 35 bp, Artificial Sequence
  primer
aaaataggcttgcattgtatgtcctcctggacttc

SEQ ID NO: 5 - DNA, 39 bp, Artificial Sequence
  primer
tacccggggatcctctagcaataactccgtgtagggtga

SEQ ID NO: 6 - DNA, 34 bp, Artificial Sequence
  primer
tgctctagaatttgatccgtttttctaaaggttg

SEQ ID NO: 7 - DNA, 35 bp, Artificial Sequence
  primer
tcaaattctagagcaattcattgacgtacaaagtg

SEQ ID NO: 8 - DNA, 37 bp, Artificial Sequence
  primer
tgcaggtcgactctagctgtggccatccttgacggga

SEQ ID NO: 9 - DNA, 362 bp, Corynebacterium glutamicum ATCC13869
agatcgtttagatccgaaggaaaacgtcgaaaagcaatttgcttttcgacgccccaccccgcgcgttttagcgtgtcagtaggcgcgtagggtaagtggggtagcggcttgttagatatcttgaaatcggctttcaacagcattgatttcgatgtatttagctggccgttaccctgcgaatgtccacagggtagctggtagtttgaaaatcaacgccgttgcccttaggattcagtaactggcacattttgtaatgcgctagatctgtgtgctcagtcttccaggctgcttatcacagtgaaagcaaaaccaattcgtggctgcgaaagtcgtagccaccacgaagtccaggaggacataca

SEQ ID NO: 10 - DNA, 2849 bp, Escherichia coli MG1655
  CDS (1)..(1323)
  CDS (1395)..(2849)
atgcaagcctattttgaccagctcgatcgcgttcgttatgaaggctcaaaatcctcaaacccgttagcattccgtcactacaatcccgacgaactggtgttgggtaagcgtatggaagagcacttgcgttttgccgcctgctactggcacaccttctgctggaacggggcggatatgtttggtgtgggggcgtttaatcgtccgtggcagcagcctggtgaggcactggcgttggcgaagcgtaaagcagatgtcgcatttgagtttttccacaagttacatgtgccattttattgcttccacgatgtggatgtttcccctgagggcgcgtcgttaaaagagtacatcaataattttgcgcaaatggttgatgtcctggcaggcaagcaagaagagagcggcgtgaagctgctgtggggaacggccaactgctttacaaaccctcgctacggcgcgggtgcggcgacgaacccagatcctgaagtcttcagctgggcggcaacgcaagttgttacagcgatggaagcaacccataaattgggcggtgaaaactatgtcctgtggggcggtcgtgaaggttacgaaacgctgttaaataccgacttgcgtcaggagcgtgaacaactgggccgctttatgcagatggtggttgagcataaacataaaatcggtttccagggcacgttgcttatcgaaccgaaaccgcaagaaccgaccaaacatcaatatgattacgatgccgcgacggtctatggcttcctgaaacagtttggtctggaaaaagagattaaactgaacattgaagctaaccacgcgacgctggcaggtcactctttccatcatgaaatagccaccgccattgcgcttggcctgttcggttctgtcgacgccaaccgtggcgatgcgcaactgggctgggacaccgaccagttcccgaacagtgtggaagagaatgcgctggtgatgtatgaaattctcaaagcaggcggtttcaccaccggtggtctgaacttcgatgccaaagtacgtcgtcaaagtactgataaatatgatctgttttacggtcatatcggcgcgatggatacgatggcactggcgctgaaaattgcagcgcgcatgattgaagatggcgagctggataaacgcatcgcgcagcgttattccggctggaatagcgaattgggccagcaaatcctgaaaggccaaatgtcactggcagatttagccaaatatgctcaggaacatcatttgtctccggtgcatcagagtggtcgccaggaacaactggaaaatctggtaaaccattatctgttcgacaaataacggctaactgtgcagtccgttggcccggttatcggtagcgataccgggcatttttttaaggaacgatcgatatgtatatcgggatagatcttggcacctcgggcgtaaaagttattttgctcaacgagcagggtgaggtggttgctgcgcaaacggaaaagctgaccgtttcgcgcccgcatccactctggtcggaacaagacccggaacagtggtggcaggcaactgatcgcgcaatgaaagctctgggcgatcagcattctctgcaggacgttaaagcattgggtattgccggccagatgcacggagcaaccttgctggatgctcagcaacgggtgttacgccctgccattttgtggaacgacgggcgctgtgcgcaagagtgcactttgctggaagcgcgagttccgcaatcgcgggtgattaccggcaacctgatgatgcccggatttactgcgcctaaattgctatgggttcagcggcatgagccggagatattccgtcaaatcgacaaagtattattaccgaaagattacttgcgtctgcgtatgacgggggagtttgccagcgatatgtctgacgcagctggcaccatgtggctggatgtcgcaaagcgtgactggagtgacgtcatgctgcaggcttgcgacttatctcgtgaccagatgcccgcattatacgaaggcagcgaaattactggtgctttgttacctgaagttgcgaaagcgtggggtatggcgacggtgccagttgtcgcaggcggtggcgacaatgcagctggtgcagttggtgtgggaatggttgatgctaatcaggcaatgttatcgctggggacgtcgggggtctattttgctgtcagcgaagggttcttaagcaagccagaaagcgccgtacatagcttttgccatgcgctaccgcaacgttggcatttaatgtctgtgatgctgagtgcagcgtcgtgtctggattgggccgcgaaattaaccggcctgagcaatgtcccagctttaatcgctgcagctcaacaggctgatgaaagtgccgagccagtttggtttctgccttatctttccggcgagcgtacgccacacaataatccccaggcgaagggggttttctttggtttgactcatcaacatggccccaatgaactggcgcgagcagtgctggaaggcgtgggttatgcgctggcagatggcatggatgtcgtgcatgcctgcggtattaaaccgcaaagtgttacgttgattgggggcggggcgcgtagtgagtactggcgtcagatgctggcggatatcagcggtcagcagctcgattaccgtacggggggggatgtggggccagcactgggcgcagcaaggctggcgcagatcgcggcgaatccagagaaatcgctcattgaattgttgccgcaactaccgttagaacagtcgcatctaccagatgcgcagcgttatgccgcttatcagccacgacgagaaacgttccgtcgcctctatcagcaacttctgccattaatggcgtaa

SEQ ID NO: 11 - protein, 440 aa, Escherichia coli MG1655
MQAYFDQLDRVRYEGSKSSNPLAFRHYNPDELVLGKRMEEHLRFAACYWHTFCWNGADMFGVGAFNRPWQQPGEALALAKRKADVAFEFFHKLHVPFYCFHDVDVSPEGASLKEYINNFAQMVDVLAGKQEESGVKLLWGTANCFTNPRYGAGAATNPDPEVFSWAATQVVTAMEATHKLGGENYVLWGGREGYETLLNTDLRQEREQLGRFMQMVVEHKHKIGFQGTLLIEPKPQEPTKHQYDYDAATVYGFLKQFGLEKEIKLNIEANHATLAGHSFHHEIATAIALGLFGSVDANRGDAQLGWDTDQFPNSVEENALVMYEILKAGGFTTGGLNFDAKVRRQSTDKYDLFYGHIGAMDTMALALKIAARMIEDGELDKRIAQRYSGWNSELGQQILKGQMSLADLAKYAQEHHLSPVHQSGRQEQLENLVNHYLFDK

SEQ ID NO: 12 - protein, 484 aa, Escherichia coli MG1655
MYIGIDLGTSGVKVILLNEQGEVVAAQTEKLTVSRPHPLWSEQDPEQWWQATDRAMKALGDQHSLQDVKALGIAGQMHGATLLDAQQRVLRPAILWNDGRCAQECTLLEARVPQSRVITGNLMMPGFTAPKLLWVQRHEPEIFRQIDKVLLPKDYLRLRMTGEFASDMSDAAGTMWLDVAKRDWSDVMLQACDLSRDQMPALYEGSEITGALLPEVAKAWGMATVPVVAGGGDNAAGAVGVGMVDANQAMLSLGTSGVYFAVSEGFLSKPESAVHSFCHALPQRWHLMSVMLSAASCLDWAAKLTGLSNVPALIAAAQQADESAEPVWFLPYLSGERTPHNNPQAKGVFFGLTHQHGPNELARAVLEGVGYALADGMDVVHACGIKPQSVTLIGGGARSEYWRQMLADISGQQLDYRTGGDVGPALGAARLAQIAANPEKSLIELLPQLPLEQSHLPDAQRYAAYQPRRETFRRLYQQLLPLMA

SEQ ID NO: 13 - DNA, 1485 bp, Corynebacterium glutamicum ATCC13869
  CDS (1)..(1485)
atgcaaaccattcagctactcaccaaagcaggacttttagtagacgcactttcggcagggccaaatactcattctgagctggcaaaacagttaaatgagccgagatcgtcaatctatcgaataacgtcttcgttagaggaagtcgggtacgtcaacatcaccagcagtggcttgttagggcttggcgtaaacatcctccacctgggcgaaagtgccgttgacgccctgcttaacagaactttattgcgggaaaaattaggctggctccgcgatcagctgggcatgaccgctttcttttgcaccctccaagatgaccgcatcatcagtctggattggcaggagggcgcagatattgatctgatttacctcgcccctggccgcacgctcccgtcccaaaaaggtgcagtctcccatgtgctccagggcaaagacctgcgcaaagggtggagtattgatcacggcgagctcaccgttggagtgtcatccttagctgtcgcggtgaaaaacgctaacggcgacgtcttaggtgcagtggcggtagctgggctgagtgcaagcgttgagagcaaaatcgacaccatccgggacacgttgaaggaaactgcgtgcgcaatcgcaaacatgccgccagccaaaacgcaggaattcgatccatcacgaatcaaggaacccaattcaccttcggtaatcaccaaagcggcaacgctcatggatgtgctccgcactgaaggtcccaccaactccgctcgcctagctgaggtgctgggggagccgatcagttcggtgtacagaatgctccacaccttaaccgcgatcgggtgggttgagcaggacggaaagcgcggctcctatcgcgttggcctagccatgctcacacttgccgaatcgcaattgcgccatatggatctccgcaagatcgccgcactgaccatgcggaaaattcacgcactcactggtgaaaccacatttttgtgtgtccgccacggcattcgcgcggtgtgcatcgagcgagttgatggcgatcgcgtgaatagtcgagttctccaattgggaacctcgctgccccttcatgtcggtgccgcaccgcgcgcgcttctcgcttttgagggacgccgggcctgggaaacgtatgccacaaacttaggattcgagggccacaactggtctaaaggtccgtccagggccgagctgttccagcacttggatgaggaccgtgacaagggattttgcctggtagacaatgaaattactcccggaatcgctgctgtgggagcacccatttacaaccaccgtggtgaagtcgtggcaagcctgtccatgagtggactgcgggacggcatcctcagcgataccaccgactactcggccgtggaactgatcctgcaggggtctgcggagatttcccaagcgctgggagcggccattgagcacaacgggggcaaccaaaaactaccccaggtaacccctctgagcattgtggtttaa

SEQ ID NO: 14 - protein, 494 aa, Corynebacterium glutamicum ATCC13869
MQTIQLLTKAGLLVDALSAGPNTHSELAKQLNEPRSSIYRITSSLEEVGYVNITSSGLLGLGVNILHLGESAVDALLNRTLLREKLGWLRDQLGMTAFFCTLQDDRIISLDWQEGADIDLIYLAPGRTLPSQKGAVSHVLQGKDLRKGWSIDHGELTVGVSSLAVAVKNANGDVLGAVAVAGLSASVESKIDTIRDTLKETACAIANMPPAKTQEFDPSRIKEPNSPSVITKAATLMDVLRTEGPTNSARLAEVLGEPISSVYRMLHTLTAIGWVEQDGKRGSYRVGLAMLTLAESQLRHMDLRKIAALTMRKIHALTGETTFLCVRHGIRAVCIERVDGDRVNSRVLQLGTSLPLHVGAAPRALLAFEGRRAWETYATNLGFEGHNWSKGPSRAELFQHLDEDRDKGFCLVDNEITPGIAAVGAPIYNHRGEVVASLSMSGLRDGILSDTTDYSAVELILQGSAEISQALGAAIEHNGGNQKLPQVTPLSIVV

SEQ ID NO: 15 - DNA, 798 bp, Sphingomonas elodea
  CDS (1)..(798)
atgtcgcaagccgatctccagcaggggccgattccggccgcccagcgcgccgtctatccgagcctgaagggcaagcgggtcctgataaccggcggtggttcgggcatcggcgccgggttggtcgaaggcttcgtccgccagggcgcggacgtgaccttcttcgacatcgccgaggcggattcgcaggcgctggtcgccagcctgaccgacgcggcgatcgcgccgcgcttctatcgtgtcgatctcaccgacattcccgccgcgcaggcgcaggtgcaggcgctgatcgaggccgagggcggcttcgacgtgctgctgaacaacgccgccaatgacgatcgccacacgatcgagcaggtgaccccggaatattgggacaaccgcctcaacgtgaacctgcgccaccagttcttcctggcgcaggcggtgattccggcgatgaaggccaagcgcgccggcgtgatcatcaacctcggctcgatctcgtggcacctcgccctggaggagctgacgctctaccagaccgccaaggcggcgatcgagggcctgacccgcagcctggcgcgcgagctgggcccggacggcatccgctcggtctgcatcgtccccggcaacgtcaagacgccgcgccagatgaagtggtacacgcccgagggcgaggccgagatcgtcaaggcgcagtgcctgcccggccgcctggtgccggacgacatcgccgcgctggcgctgttccttgcatccgacgatgcccggctgataacgagccacgaattcttcgtggatgcaggctggagataa

SEQ ID NO: 16 - protein, 265 aa, Sphingomonas elodea
MSQADLQQGPIPAAQRAVYPSLKGKRVLITGGGSGIGAGLVEGFVRQGADVTFFDIAEADSQALVASLTDAAIAPRFYRVDLTDIPAAQAQVQALIEAEGGFDVLLNNAANDDRHTIEQVTPEYWDNRLNVNLRHQFFLAQAVIPAMKAKRAGVIINLGSISWHLALEELTLYQTAKAAIEGLTRSLARELGPDGIRSVCIVPGNVKTPRQMKWYTPEGEAEIVKAQCLPGRLVPDDIAALALFLASDDARLITSHEFFVDAGWR

SEQ ID NO: 17 - DNA, 894 bp, Sphingomonas elodea
  CDS (1)..(894)
atgaccgacaaggtggtggtttcggcgccggagagcgtgtgggggctcagcgccccgcttctcgaaggcccggtatgggtggagcgcgatgccgcgctttggttcgtcgacatcaagagccacaagatccaccgctatgatcccgccaccggcgacaaggcgagctgggacgcgccggcgcaggtgggcttcgcgctgccggcggcgagcggcggcttcgtcgcggggctgcagaccgggctcgccaggttcgatccgacggacggcagcttcgtgcccctggtcgatcccgaacccgaactgcccggcaaccggctgaacgacggcaccgtcgattcggaaggccgcctgtggttcggcacgatggacgacggcgagagcgcggccaccggcaccatctatcgcctggcagcggacggcagctgcgtgccctccagccccaaggtatcgatcaccaacggcccggcggtctcgcccgacggcaagacgctctaccatgtcgatacgctcggcgcggtggtctatgcctgcgacatcgatccggacggcgcgctggtgaaccgccgcgagttcgtgcgcatcgccgagggcgaaggcttcccggacggcccgtgcgtcgacagcgagggctatgtgtgggtgagcctgtacgtcggctcggaggtgcgtcgctactcgcctgcgggcgagctggtcgagacggtgcccttccccgtcgatgcgatcaccaagatcgcgttcggcggcccggacctgaagacggtcttcgccaccaccgcgaacaagcacctttcggccgaagacaaggccgcacggccgagttcgggcgacctgttccgcttccgcgtgacggtggccggtcagccgaccgcgatgatccgcatcggggcctga

SEQ ID NO: 18 - protein, 297 aa, Sphingomonas elodea
MTDKVVVSAPESVWGLSAPLLEGPVWVERDAALWFVDIKSHKIHRYDPATGDKASWDAPAQVGFALPAASGGFVAGLQTGLARFDPTDGSFVPLVDPEPELPGNRLNDGTVDSEGRLWFGTMDDGESAATGTIYRLAADGSCVPSSPKVSITNGPAVSPDGKTLYHVDTLGAVVYACDIDPDGALVNRREFVRIAEGEGFPDGPCVDSEGYVWVSLYVGSEVRRYSPAGELVETVPFPVDAITKIAFGGPDLKTVFATTANKHLSAEDKAARPSSGDLFRFRVTVAGQPTAMIRIGA

SEQ ID NO: 19 - DNA, 1968 bp, Escherichia coli MG1655
  CDS (1)..(1968)
atgaccattgagaaaattttcaccccgcaggacgacgcgttttatgcggtgatcacccacgcggcggggccgcagggcgctctgccgctgaccccgcagatgctgatggaatctcccagcggcaacctgttcggcatgacgcagaacgccgggatgggctgggacgccaacaagctcaccggcaaagaggtgctgattatcggcactcagggcggcatccgcgccggagacggacgcccaatcgcgctgggctaccacaccgggcattgggagatcggcatgcagatgcaggcggcggcgaaggagatcacccgcaatggcgggatcccgttcgcggccttcgtcagcgatccgtgcgacgggcgctcgcagggcacgcacggtatgttcgattccctgccgtaccgcaacgacgcggcgatcgtgtttcgccgcctgatccgctccctgccgacgcggcgggcggtgatcggcgtagcgacctgcgataaagggctgcccgccaccatgattgcgctggccgcgatgcacgacctgccgactattctggtgccgggcggggcgacgctgccgccgaccgtcggggaagacgcgggcaaggtgcagaccatcggcgcgcgtttcgccaaccacgaactctccctgcaggaggccgccgaactgggctgtcgcgcctgcgcctcgccgggcggcgggtgtcagttcctcggcacggcgggcacctcgcaggtggtcgcggaggcgctgggtctggcgctgccgcactccgcgctggcgccgtccgggcaggcggtgtggctggagatcgcccgccagtcggcgcgcgcggtcagcgagctggatagccgcggcatcaccacgcgggatatcctctccgataaagccatcgaaaacgcgatggtgatccacgcggcgttcggcggctccaccaatttactgctgcacattccggccatcgcccacgcggcgggctgcacgatcccggacgttgagcactggacgcgcatcaaccgtaaagtgccgcgtctggtgagcgtgctgcccaacggcccggactatcacccgaccgtgcgcgccttcctcgcgggcggcgtgccggaggtgatgctccacctgcgcgacctcggcctgctgcatctggacgccatgaccgtgaccggccagacggtgggcgagaaccttgaatggtggcaggcgtccgagcgccgggcgcgcttccgccagtgcctgcgcgagcaggacggcgtagagccggatgacgtgatcctgccgccggagaaggcaaaagcgaaagggctgacctcgacggtctgcttcccgacgggcaacatcgctccggaaggttcggtgatcaaggccacggcgatcgacccgtcggtggtgggcgaagatggcgtataccaccacaccggccgggtgcgggtgtttgtctcggaagcgcaggcgatcaaggcgatcaagcgggaagagattgtgcagggcgatatcatggtggtgatcggcggcgggccgtccggcaccggcatggaagagacctaccagctcacctccgcgctaaagcatatctcgtggggcaagacggtgtcgctcatcaccgatgcgcgcttctcgggcgtgtcgacgggcgcctgcttcggccacgtgtcgccggaggcgctggcgggcgggccgattggcaagctgcgcgataacgacatcatcgagattgccgtggatcgtctgacgttaactggcagcgtgaacttcatcggcaccgcggacaacccgctgacgccggaagagggcgcgcgcgagctggcgcggcggcagacgcacccggacctgcacgcccacgactttttgccggacgacacccggctgtgggcggcactgcagtcggtgagcggcggcacctggaaaggctgtatttatgacaccgataaaattatcgaggtaattaacgccggtaaaaaagcgctcggaatttaa

SEQ ID NO: 20 - protein, 655 aa, Escherichia coli MG1655
MTIEKIFTPQDDAFYAVITHAAGPQGALPLTPQMLMESPSGNLFGMTQNAGMGWDANKLTGKEVLIIGTQGGIRAGDGRPIALGYHTGHWEIGMQMQAAAKEITRNGGIPFAAFVSDPCDGRSQGTHGMFDSLPYRNDAAIVFRRLIRSLPTRRAVIGVATCDKGLPATMIALAAMHDLPTILVPGGATLPPTVGEDAGKVQTIGARFANHELSLQEAAELGCRACASPGGGCQFLGTAGTSQVVAEALGLALPHSALAPSGQAVWLEIARQSARAVSELDSRGITTRDILSDKAIENAMVIHAAFGGSTNLLLHIPAIAHAAGCTIPDVEHWTRINRKVPRLVSVLPNGPDYHPTVRAFLAGGVPEVMLHLRDLGLLHLDAMTVTGQTVGENLEWWQASERRARFRQCLREQDGVEPDDVILPPEKAKAKGLTSTVCFPTGNIAPEGSVIKATAIDPSVVGEDGVYHHTGRVRVFVSEAQAIKAIKREEIVQGDIMVVIGGGPSGTGMEETYQLTSALKHISWGKTVSLITDARFSGVSTGACFGHVSPEALAGGPIGKLRDNDIIEIAVDRLTLTGSVNFIGTADNPLTPEEGARELARRQTHPDLHAHDFLPDDTRLWAALQSVSGGTWKGCIYDTDKIIEVINAGKKALGI

SEQ ID NO: 21 - DNA, 1113 bp, Sphingomonas elodea
  CDS (1)..(1113)
atgctgcctgccgatcatgcgcaggcgattctggtcggccgtgtgcagaccccggcgggcccgagccccgttctcctccgcgatggccaggtgatcgacgtttcggcgatcgcgccgaccgtcgccgacctgctggaacgcgacgacatcgcgacgctgagcggcacggtgctgtgcagcgtcgacgcgctcggcaccgagtcggcgccgcaggtgctggctccggtcgacctgcagtgcgtgaaggccgccggcgtcaccttcgccgtctcggcgctggagcgcgtgatcgaggaacgcgcccgcggcgattccgccaaggccgccgagattcgcggcgacctcgaagccaaggtgggttcgggcatccgctcggtcgtccccggtaccgccgaggccgcggcgctcaaggccgcgctgatcgaggcgggcatgtggtcgcaatatctcgaagtggcgatcgggccggacgcggaggtgttcaccaaggcgccggttctgtcggcgatgggctggggcgccgagatcggcatccgctcggacagcgactggaacaatccggagccggaagtggtgctggtggtcgaccggaatggtgcgatcaagggcgcgacgctcggcaacgacgtcaacctgcgcgacttcgagggccgcagcgcgctgctgctgggcaaggcgaaggacaacaatgcctctaccgcgatcggcccgttcatccgcctgttcgatgacggcttcacgatggacgacgtgcgtagcgcggtggtcgacctcaccatcgacgggccggagggctatcgcctctcgggcaccaacaagatgagcgagatcagccgagatccgaccgagctcgtgcgccagacgctgagcgagcaccagtatccggacggcttcgcgctgttcctcggcacgctgttcgcgccggtgcaggatcgcgaccatcccggccgcggcttcactcacaagcccggcgatattgtccgcatttccacgccgaagctcggcacgctcgtcaaccgcgtcaccacgtccaaggccgccgcgccctggacgttcggcatccgcgatctgatgcgcaatctcgccgcccgcggccttctctcgcattcctaa

SEQ ID NO: 22 - protein, 370 aa, Sphingomonas elodea
MLPADHAQAILVGRVQTPAGPSPVLLRDGQVIDVSAIAPTVADLLERDDIATLSGTVLCSVDALGTESAPQVLAPVDLQCVKAAGVTFAVSALERVIEERARGDSAKAAEIRGDLEAKVGSGIRSVVPGTAEAAALKAALIEAGMWSQYLEVAIGPDAEVFTKAPVLSAMGWGAEIGIRSDSDWNNPEPEVVLVVDRNGAIKGATLGNDVNLRDFEGRSALLLGKAKDNNASTAIGPFIRLFDDGFTMDDVRSAVVDLTIDGPEGYRLSGTNKMSEISRDPTELVRQTLSEHQYPDGFALFLGTLFAPVQDRDHPGRGFTHKPGDIVRISTPKLGTLVNRVTTSKAAAPWTFGIRDLMRNLAARGLLSHS

SEQ ID NO: 23 - DNA, 1467 bp, Bacillus subtilis
  CDS (1)..(1467)
atgtctgtgatcacggaacaaaacacgtacctcaactttattaacggagagtgggttaagtctcaatcaggcgatatggtcaaagtcgaaaaccctgccgatgtgaatgatattgtcggatatgtacagaattcaacggctgaagatgtggaacgtgccgtcaccgccgccaatgaagccaaaacggcttggagaaagctgacgggtgccgagcgcggccaatacttatacaaaacagcggatatcatggagcagcgcttggaggaaatcgccgcctgtgcaacgcgtgaaatgggtaaaacattgccggaagcgaagggagaaacagcccgggggattgccattctgcgctattacgccggagagggcatgcgaaaaacgggtgacgtcattccgtctactgacaaagacgcgctcatgtttaccacccgtgttccgctcggtgtggtcggtgtgatttctccgtggaacttcccagtggcgattccgatttggaaaatggcgccggcattggtatacggcaataccgttgtcatcaaaccggcgacagaaacagctgtgacatgcgcgaagatcattgcctgctttgaggaagcggggctcccggcaggggtcatcaatttggtgacaggcccgggttctgttgtcgggcaggggcttgctgagcatgacggtgtaaacgccgttacgtttaccggttcaaatcaagtcggaaaaatcatcgggcaagccgctttagcgaggggagccaaatatcagcttgagatgggcggcaaaaaccctgtcatcgtagctgatgacgctgaccttgaagctgcggcagaagctgtcataacgggggccttccgttcaaccggccagaaatgcaccgcgacaagccgtgtcatcgtacaaagcggaatttacgagcgctttaaagaaaaactgctccagcgcacaaaagatattacaatcggagacagcttaaaagaggatgtctggatgggaccgatagccagcaagaatcagcttgataactgcctgtcatacattgagaaaggcaaacaggagggcgcttcccttttaataggaggagaaaagctggagaacggaaagtatcaaaacggctattatgttcagcctgccatctttgacaatgtgacatctgagatgacaattgcccaggaggaaattttcggtccggtgatcgccttgatcaaggtggactcgatagaggaggcgctgaacatcgccaatgatgtgaagttcggtttaagtgcatccatcttcacggaaaacatcggccgaatgctttctttcattgatgaaatcgatgccgggctggttcggatcaatgcagaaagcgcaggtgttgagctgcaggcgccttttggcggcatgaagcagtcgagctcccactcccgagaacagggtgaggcagcgaaggactttttcacagcgatcaaaactgtttttgtgaagccgtaa

SEQ ID NO: 24 - protein, 488 aa, Bacillus subtilis
MSVITEQNTYLNFINGEWVKSQSGDMVKVENPADVNDIVGYVQNSTAEDVERAVTAANEAKTAWRKLTGAERGQYLYKTADIMEQRLEEIAACATREMGKTLPEAKGETARGIAILRYYAGEGMRKTGDVIPSTDKDALMFTTRVPLGVVGVISPWNFPVAIPIWKMAPALVYGNTVVIKPATETAVTCAKIIACFEEAGLPAGVINLVTGPGSVVGQGLAEHDGVNAVTFTGSNQVGKIIGQAALARGAKYQLEMGGKNPVIVADDADLEAAAEAVITGAFRSTGQKCTATSRVIVQSGIYERFKEKLLQRTKDITIGDSLKEDVWMGPIASKNQLDNCLSYIEKGKQEGASLLIGGEKLENGKYQNGYYVQPAIFDNVTSEMTIAQEEIFGPVIALIKVDSIEEALNIANDVKFGLSASIFTENIGRMLSFIDEIDAGLVRINAESAGVELQAPFGGMKQSSSHSREQGEAAKDFFTAIKTVFVKP

SEQ ID NO: 25 - DNA, 3481 bp, Corynebacterium glutamicum 2256 (ATCC 13869)
  CDS (1437)..(3035)
gatcttgccgatttcggcaggatcaatgtcggcgtgaatgatcttggcatcaggtgcgaaagtgtcaacgtcaccggtgacgcggtcatcaaagcgggagccgatagcaatcagcaggtcgctgcgctgcagtgcaccaacagcggacacagtgccatgcatgcctggcatacccatgtgcagctcgtgggactctgggaaggttcccagcgccatcaatgtggtgacaactggaatgccggtgtgctcagcgaacgcacgaagctcttcgtgggcatcagccttgataacgccgccgccaacgtaaaggacaggcttcttagactcaccgatcagtttgacagcctgctcaatctgtcgagcatgcggtgttgaaactgggcggtagcctggcaggtcgatctttggtggccagacgaaatccaattcagcgttctgaacatccttggggatatccactagaacaggaccagggcgaccagtaatcgcgaggtggaatgcctcagccaatgcctgtggaatgtcgttggggttggtgaccatgaagttgtgcttggtcactggcatggtgatgccgcggatatcggcttcctggaaagcatcggtacccagcaggctacttccgacctggccggtgatggcaaccatgggaacggagtccaagtttgcatcagcgattggggtaaccaagttggttgcgcctgggccagaggttgcaatgcagacgccaacgcgtccagtaacctgcgcgtagccggttgctgcgtggcctgcgccctgctcgtggcgcactaggacgtggcgcacctttgtggaggaatagagcgggtcatacaccggtagcaccgcaccaccaggaataccgaacacgatgtcggcgttaagctcctcgagcgatcgaacaattgcctgtgcacctgtcatccgctcaggggcggcggatcgaccacggcttgcaaccgtggcgggagtgggctgttgagaagctgccacattcacgactttctggctcctttactaaataaggattttcacaggacccgtccaagccaagccgatttcaactcagcctaaagacaaagccctcatttaaaattgttccgacgcggatgcgtgtgcacgcagtgcgacagatgtctgttgcaaagttggctacttgggtcataaccaacaagaaagccctcgttccaacactgtggtgagtgttgtcgagggcgcttgacgagacgacttggaaggccgttacggcaggcgccgcgcggttactactacaagtcgaataatggtcatggtgtgtcatgctacacacatcgagtttccaattccacaacgcacgaaaattcccacccccaaaactcccccacttcggttaaggaatcaggattctcacaaagttcaggcaggctcccgctacttttcagcgctaatcttggctcatgattttaggcgtacccattcaatatttgctctattcattgtggaattggattgtcgataccggttttgatgtagcaattatcctggtcttggcgtttttgattccacgtatcggccgactggccatgcgtattatcaagcagcgagtggagtctgcagccgatgcggacaccactaagaaccagctcgcgttcgctggcgttggcgtttatatcgcgcaaattgtggcgtttttcatgcttgccgtctccgcgatgcaggcttttggtttctctctcgcgggcgctgcgattccggcaaccattgcgtcagctgccattggtcttggtgcgcagtcgattgttgcggacttcttggccggatttttcatcctgacggaaaagcaattcggcgtgggtgactgggtgcgctttgagggcaacggcatcgttgttgaaggcaccgtcattgagatcaccatgcgcgcgaccaaaattcgcacgattgcacaagagaccgtgatcatcccgaactccacggcgaaagtgtgcatcaacaattctaataactggtcgcgtgcggttgtcgttattccgatccccatgttgggttctgaaaacatcacagatgtcatcgcgcgctctgaagctgcgactcgtcgcgcacttggccaggagaaaatcgcaccggaaatcctcggtgaactcgatgtgcacccagccacggaagtcacaccgccaacggtggtcggcatgccgtggatggtcaccatgcgtttcctcgtgcaagtcaccgccggcaatcaatggctggtcgaacgcgccatccgcacagaaatcatcaacgaattctgggaagaatacggcagcgcaaccactacatcgggaaccctcattgattccttacacgttgagcatgaagagccaaagacctcgcttatcgacgcctccccccaggctcttaaggaaccgaagccggaggctgcggcgacggttgcatcgctagctgcatcgtctaacgacgatgcagacaatgcagacgcctcggcgatcaatgcaggcaatccagagaaggaacttgattccgatgtgctggaacaagaactctccagcgaagaaccggaagaaacagcaaaaccagatcactctctccgaggcttcttccgcactgattactacccaaatcggtggcagaagatcctgtcgtttggcggacgtgtccgcatgagcacttccctgttgttgggtgcgctgctcttgctgtcactatttaaggtcatgactgtggaaccaagtgagaattggcaaaactccagtggatggctgtcaccaagcactgccacctcaactgcggtgaccacctccgaaacttccgcgccagcaagcacgccttcgatgacagtgcccactacggtggaggagaccccaacgatggaatctagcgtcgaaacgcagcaggaaacctcaacccctgcaaccgcaacgccccagcgagccgacaccatcgaaccgaccgaggaagccacgtcgcaggaggaaacgactgcatcgcagacgcagtctccagcagtggaagcaccaaccgcggtccaagaaacagttgcgccgacgtccaccccttaggacgctgattacagacgtgtcccatttctttactactattggaaattatgagttcagacgcagaaaaggcatccgtggagctttccgaaaaatttcacccagaacgcacccatattttgggcgccgttgtttttggcctgatctcattattagtcatcggcgcagcccctcagtacctgttttggctgctcgcgctccctgtcatcttcggttactgggttctaaaatcatccacgatcgttgatgaacagggcatcaccgcaaactacgccttcaagggcaaaaaggttgtggcctgggaagacctcgcaggaatcggattcaagggtgcccgcactttcgctcgcaccacctccgatgcagaagtcaccctccccggcgtcaccttcaactcccttccccgccttgaagctgcttcccacggccgcatccccgatgcgatc

SEQ ID NO: 26 - protein, 533 aa, Corynebacterium glutamicum 2256 (ATCC 13869)
MILGVPIQYLLYSLWNWIVDTGFDVAIILVLAFLIPRIGRLAMRIIKQRVESAADADTTKNQLAFAGVGVYIAQIVAFFMLAVSAMQAFGFSLAGAAIPATIASAAIGLGAQSIVADFLAGFFILTEKQFGVGDWVRFEGNGIVVEGTVIEITMRATKIRTIAQETVIIPNSTAKVCINNSNNWSRAVVVIPIPMLGSENITDVIARSEAATRRALGQEKIAPEILGELDVHPATEVTPPTVVGMPWMVTMRFLVQVTAGNQWLVERAIRTEIINEFWEEYGSATTTSGTLIDSLHVEHEEPKTSLIDASPQALKEPKPEAAATVASLAASSNDDADNADASAINAGNPEKELDSDVLEQELSSEEPEETAKPDHSLRGFFRTDYYPNRWQKILSFGGRVRMSTSLLLGALLLLSLFKVMTVEPSENWQNSSGWLSPSTATSTAVTTSETSAPASTPSMTVPTTVEETPTMESSVETQQETSTPATATPQRADTIEPTEEATSQEETTASQTQSPAVEAPTAVQETVAPTSTP

SEQ ID NO: 27 - DNA, 44 bp, Artificial Sequence
  primer
tacccggggatcctctaggcgctgaactcacaattccgattagt

SEQ ID NO: 28 - DNA, 50 bp, Artificial Sequence
  primer
atattcagcgggttctggaaccacattgggtggaactctagattccaaga

SEQ ID NO: 29 - DNA, 50 bp, Artificial Sequence
  primer
tcttggaatctagagttccacccaatgtggttccagaacccgctgaatat

SEQ ID NO: 30 - DNA, 41 bp, Artificial Sequence
  primer
tgcaggtcgactctaggggcaggttttggtgtggcaggatg

SEQ ID NO: 31 - DNA, 39 bp, Artificial Sequence
  primer
ggagccttcgcctctatgaccattgagaaaattttcacc

SEQ ID NO: 32 - DNA, 40 bp, Artificial Sequence
  primer
tggttcttggaatctttaaattccgagcgcttttttaccg

SEQ ID NO: 33 - DNA, 37 bp, Artificial Sequence
  primer
attgggtggaactctaaattcctgtgaagtagctgat

SEQ ID NO: 34 - DNA, 26 bp, Artificial Sequence
  primer
agaggcgaaggctccttgaataggta

SEQ ID NO: 35 - DNA, 1383 bp, Corynebacterium glutamicum ATCC13869
atggctctggttcttggaatcgatagttccacccaatcctgcaaggctttgcttgtcgacgccgccagcggccgcattatcgacgaaggccgcgcgagtcacccgagcgggtcggaggtagatccacgtgcgtggatcgctgcgctggatcaagctaccgaggggttgctagaacgtgcggatgctgtgtctattgcaggccagcagcacggcatggtggcgttggatgaaaacgatgaaatcgttcgcccggcgttgttgtggaatgacactcgttctgcccaggctgcgttggatctcaatgaggagatcggcggcgatcaggctgcggtagatgccacgggaagtgtgtatgttgcttctttaactgccaccaagatgcggtggatgcgtgatcatgagccagaaaatgcagcgcgtacagcgtcggtgatgttgcctcatgatttcctcacctggcatttgatgggacgtggccgcaaagtcactgatcatggtgatgcttccggaacgggctactacagcactcgtgatcgtgcgtggcgcaccgatctagctgccttggcgctgggccatgaggtggaacttcctgaactcctggctccgaatgagattgcgggaacaactccaggtggtgtgaaagttgctgcaggcacgggcgataatgctgcggctgcgcttggccttgatttgcatccaggcgatgtcagcgtgtcgatcggcacctcaggcgttgccggcatgactgttcaaaacagcgtccacgatccgtctggtctggtcactggttttgccgatgccacgggtgcgtatttcccgctggcctgcacgctcaatggcgcaccggtgctggaattcggccgccgcattctgggcgtggaatgggaagagttcgatgcgcttgcgctagctgctcaacccggttcaggtggagtaacgttccagccttatttggagggcgagcgtacgccgaatcgtcccgcagcacgtggcgttttggctggactaaacagtgcaactacccgcgaggattttgcccgcgcaactgttgaaggcttgttgttggcgttagatgatgctgtaacggctctggttgaggccacgggggtgcccgttcagcgcattcaactcatcggtggcggcgcgcgttcacgggcagttcgtgagatcgctcctgagattttcggccatgagattgtggttccagaacccgctgaatatgtggcgttgggtgcagctcgtcaggcggcatgggcgctgtcgggtgaggccacgccaccgcagtggccaacccttggttcagatccgcaccgcgcgcccaaaaacactgagctgagcacgcgttatgcgaagctgcgtgatgcaacgcagggttggtactag

SEQ ID NO: 36 - protein, 460 aa, Corynebacterium glutamicum ATCC13869
MALVLGIDSSTQSCKALLVDAASGRIIDEGRASHPSGSEVDPRAWIAALDQATEGLLERADAVSIAGQQHGMVALDENDEIVRPALLWNDTRSAQAALDLNEEIGGDQAAVDATGSVYVASLTATKMRWMRDHEPENAARTASVMLPHDFLTWHLMGRGRKVTDHGDASGTGYYSTRDRAWRTDLAALALGHEVELPELLAPNEIAGTTPGGVKVAAGTGDNAAAALGLDLHPGDVSVSIGTSGVAGMTVQNSVHDPSGLVTGFADATGAYFPLACTLNGAPVLEFGRRILGVEWEEFDALALAAQPGSGGVTFQPYLEGERTPNRPAARGVLAGLNSATTREDFARATVEGLLLALDDAVTALVEATGVPVQRIQLIGGGARSRAVREIAPEIFGHEIVVPEPAEYVALGAARQAAWALSGEATPPQWPTLGSDPHRAPKNTELSTRYAKLRDATQGWY

SEQ ID NO: 37 - DNA, 1437 bp, Caulobacter crescentus CB15
atgaccgacaccctgcgccattacatcggcggcgaacgcgtcgcggccgacgccccggccgagagcctgaacccgtccaacaccaacgacgtcgtcgccaaggtcccgatgggcggccaggccgaggtcgacgccgccgtcgacgccgcgcgcaaggccttcccggcctgggccgacgcctcgccggaggtccgctcggacctcttggacaaggtcggttcgaccatcatcgcccgcagcgccgacatcggccgcctgctggcccgcgaagagggcaagaccctggcggaaggcatcggcgagaccgtccgcgccggccgcatcttcaagtacttcgccggtgaagccctgcgccgtcacggccagaacctggaaagcacccgtccgggcgtcgagatccagacctatcgtcaggccgtgggcgtctatggcctgatcacgccctggaacttcccgatcgccatcccggcctggaaggccgccccggcgctcgccttcggcaacaccgtggtgatcaagccggccggcccgacgcccgccaccgccaacgtgctggccgacatcatggccgagtgcggcgccccggccggcgtgttcaacatgctgtttggtcgcggctcgatgggcgatgcgctgatcaagcacaaggacgtggacggcgtctcgttcaccggctcgcagggcgtgggcgcgcaggtcgccgccgccgccgtggcccgtcaggcccgcgtgcagctggagatgggcggcaagaacccgctgatcgtgctggacgacgccgacctggagcgcgcggtcgccatcgccctggacggctcgttcttcgccaccggccagcgctgcaccgccagctcgcgcctgatcgtccaggacgggattcacgacaagttcgtggccctgctggccgagaaggtcgccgccctgcgcgtgggcgacgctctggaccccaacacccagatcggcccggccgtctccgaagaccagatggagacttcgtaccgctatatcgacatcgctgcctccgaaggcggccgcgtggtcaccggcggcgaccgcatcaagctcgacaatccgggctggtacgtgcgtccgaccctgatcgccgacacgcaagccggcatgcggatcaacaacgaggaggtcttcggccccgtcgcctcgaccatccgcgtcaagagctacgaagaggcgctggagatcgccaacggcgtcgagttcggcctttcggccggcatcgccaccacctcgctcaagcacgcccgccacttccagcgctatgcccgcgcgggcatgaccatggtcaatctggccacggccggcgtcgactatcacgtgccgttcggcggcacgaagagcagctcgtacggcgcccgcgagcagggcttcgcggcggtcgagttcttcacccagaccaaaacctcctactcgtggtcgtaa

SEQ ID NO: 38 - protein, 478 aa, Caulobacter crescentus CB15
MTDTLRHYIGGERVAADAPAESLNPSNTNDVVAKVPMGGQAEVDAAVDAARKAFPAWADASPEVRSDLLDKVGSTIIARSADIGRLLAREEGKTLAEGIGETVRAGRIFKYFAGEALRRHGQNLESTRPGVEIQTYRQAVGVYGLITPWNFPIAIPAWKAAPALAFGNTVVIKPAGPTPATANVLADIMAECGAPAGVFNMLFGRGSMGDALIKHKDVDGVSFTGSQGVGAQVAAAAVARQARVQLEMGGKNPLIVLDDADLERAVAIALDGSFFATGQRCTASSRLIVQDGIHDKFVALLAEKVAALRVGDALDPNTQIGPAVSEDQMETSYRYIDIAASEGGRVVTGGDRIKLDNPGWYVRPTLIADTQAGMRINNEEVFGPVASTIRVKSYEEALEIANGVEFGLSAGIATTSLKHARHFQRYARAGMTMVNLATAGVDYHVPFGGTKSSSYGAREQGFAAVEFFTQTKTSYSWS

SEQ ID NO: 39 - DNA, 747 bp, Caulobacter crescentus CB15
atgtcctcagccatctatcccagcctgaagggcaagcgcgtcgtcatcaccggcggcggctcgggcatcggggccggcctcaccgccggcttcgcccgtcagggcgcggaggtgatcttcctcgacatcgccgacgaggactccagggctcttgaggccgagctggccggctcgccgatcccgccggtctacaagcgctgcgacctgatgaacctcgaggcgatcaaggcggtcttcgccgagatcggcgacgtcgacgtgctggtcaacaacgccggcaatgacgaccgccacaagctggccgacgtgaccggcgcctattgggacgagcggatcaacgtcaacctgcgccacatgctgttctgcacccaggccgtcgcgccgggcatgaagaagcgtggcggcggggcggtgatcaacttcggttcgatcagctggcacctggggcttgaggacctcgtcctctacgaaaccgccaaggccggcatcgaaggcatgacccgcgcgctggcccgggagctgggtcccgacgacatccgcgtcacctgcgtggtgccgggcaacgtcaagaccaagcgccaggagaagtggtacacgcccgaaggcgaggcccagatcgtggcggcccaatgcctgaagggccgcatcgtcccggagaacgtcgccgcgctggtgctgttcctggcctcggatgacgcgtcgctctgcaccggccacgaatactggatcgacgccggctggcgttga

SEQ ID NO: 40 - protein, 248 aa, Caulobacter crescentus CB15
MSSAIYPSLKGKRVVITGGGSGIGAGLTAGFARQGAEVIFLDIADEDSRALEAELAGSPIPPVYKRCDLMNLEAIKAVFAEIGDVDVLVNNAGNDDRHKLADVTGAYWDERINVNLRHMLFCTQAVAPGMKKRGGGAVINFGSISWHLGLEDLVLYETAKAGIEGMTRALARELGPDDIRVTCVVPGNVKTKRQEKWYTPEGEAQIVAAQCLKGRIVPENVAALVLFLASDDASLCTGHEYWIDAGWR

SEQ ID NO: 41 - DNA, 870 bp, Caulobacter crescentus CB15
atgaccgctcaagtcacttgcgtatgggatctgaaggccacgttgggcgaaggcccgatctggcatggcgacaccctgtggttcgtcgacatcaagcagcgtaaaatccacaactaccaccccgccaccggcgagcgcttcagcttcgacgcgccggatcaggtgaccttcctcgcgccgatcgtcggcgcgaccggctttgtcgtcggtctgaagaccgggattcaccgcttccacccggccacgggcttcagcctgctgctcgaggtcgaggacgcggcgctgaacaaccgccccaacgacgccacggtcgacgcgcaaggccgtctgtggttcggcaccatgcacgacggggaagagaacaatagcggctcgctctatcggatggacctcaccggcgtcgcccggatggaccgcgacatctgcatcaccaacggcccgtgcgtctcgcccgacggcaagaccttctaccacaccgacaccctggaaaagacgatctacgccttcgacctggccgaggacggcctgctgtcgaacaagcgcgtcttcgtgcagttcgccctgggcgacgatgtctatccggacggttcggtcgtcgattccgaaggctatctgtggaccgccctgtggggcggtttcggcgcggtccgcttctcgccgcaaggcgacgccgtgacgcgcatcgaactgcccgcccccaacgtcaccaagccctgcttcggcgggcctgacctgaagaccctctatttcaccaccgcccgcaagggcctgagcgacgagaccctggcccagtacccgctggccggcggtgtgttcgccgttccggtcgatgtggccggccaaccccagcatgaggtccgccttgtctaa

SEQ ID NO: 42 - protein, 289 aa, Caulobacter crescentus CB15
MTAQVTCVWDLKATLGEGPIWHGDTLWFVDIKQRKIHNYHPATGERFSFDAPDQVTFLAPIVGATGFVVGLKTGIHRFHPATGFSLLLEVEDAALNNRPNDATVDAQGRLWFGTMHDGEENNSGSLYRMDLTGVARMDRDICITNGPCVSPDGKTFYHTDTLEKTIYAFDLAEDGLLSNKRVFVQFALGDDVYPDGSVVDSEGYLWTALWGGFGAVRFSPQGDAVTRIELPAPNVTKPCFGGPDLKTLYFTTARKGLSDETLAQYPLAGGVFAVPVDVAGQPQHEVRLV

SEQ ID NO: 43 - DNA, 1788 bp, Caulobacter crescentus CB15
atgaggtccgccttgtctaaccgcacgccccgccggttccggtcccgcgattggttcgataaccccgaccatatcgacatgaccgcgctctatctggagcgcttcatgaactacgggatcacgccggaggagctgcgcagcggcaagccgatcatcggcatcgcccagaccggcagcgacatctcgccctgcaaccgcatccacctggacctggtccagcgggtgcgggacgggatccgcgacgccgggggcatccccatggagttcccggtccatccgatcttcgagaactgccgtcgcccgacggcggcgctggaccggaacctctcgtacctgggtctcgtcgagaccctgcacggctatccgatcgacgccgtggttctgaccaccggctgcgacaagaccaccccggccgggatcatggccgccaccacggtcaatatcccggccatcgtgctgtcgggcggcccgatgctggacggctggcacgagaacgagctcgtgggctcgggcaccgtgatctggcgctcgcgccgcaagctggcggccggcgagatcaccgaggaagagttcatcgaccgcgccgccagctcggcgccgtcggcgggccactgcaacaccatgggcacggcctcgaccatgaacgccgtggccgaggcgctgggcctgtcgctgaccggctgcgcggccatccccgccccctaccgcgagcgcggccagatggcctacaagaccggccagcgcatcgtcgatctggcctatgacgacgtcaaaccgctcgacatcctgaccaagcaagccttcgagaacgccatcgccctggtggcggcggccggcggctcgaccaacgcccagccgcacatcgtggccatggcccgtcacgccggcgtcgagatcaccgccgacgactggcgcgcggcctatgacatcccgctgatcgtcaacatgcagccggccggcaagtatctgggcgagcgcttccaccgagccggcggcgcgccggcggtgctgtgggagctgttgcagcaaggccgcctgcacggcgacgtgctgaccgtcaccggcaagacgatgagcgagaacctgcaaggccgcgaaaccagcgaccgcgaggtgatcttcccgtaccacgagccgctggccgagaaggccgggttcctggttctcaagggcaacctcttcgacttcgcgatcatgaagtccagcgtgatcggcgaggagttccgcaagcgctacctgtcgcagcccggccaggaaggcgtgttcgaagcccgcgccatcgtgttcgacggctcggacgactatcacaagcggatcaacgatccggccctggagatcgacgagcgctgcatcctggtgatccgcggcgcgggtccgatcggctggcccggctcggccgaggtcgtcaacatgcagccgccggatcaccttctgaagaaggggatcatgagcctgcccaccctgggcgatggccgtcagtcgggcaccgccgacagcccctcgatcctgaacgcctcgcccgaaagcgcgatcggcggcggcctgtcgtggctgcgcaccggcgacaccatccgcatcgacctcaacaccggccgctgcgacgccctggtcgacgaggcgacgatcgccgcgcgcaagcaggacggcatcccggcggttcccgccaccatgacgccctggcaggaaatctaccgcgcccacgccagtcagctcgacaccggcggcgtgctggagttcgcggtcaagtaccaggacctggcggccaagctgccccgccacaaccactga

SEQ ID NO: 44 - protein, 595 aa, Caulobacter crescentus CB15
MRSALSNRTPRRFRSRDWFDNPDHIDMTALYLERFMNYGITPEELRSGKPIIGIAQTGSDISPCNRIHLDLVQRVRDGIRDAGGIPMEFPVHPIFENCRRPTAALDRNLSYLGLVETLHGYPIDAVVLTTGCDKTTPAGIMAATTVNIPAIVLSGGPMLDGWHENELVGSGTVIWRSRRKLAAGEITEEEFIDRAASSAPSAGHCNTMGTASTMNAVAEALGLSLTGCAAIPAPYRERGQMAYKTGQRIVDLAYDDVKPLDILTKQAFENAIALVAAAGGSTNAQPHIVAMARHAGVEITADDWRAAYDIPLIVNMQPAGKYLGERFHRAGGAPAVLWELLQQGRLHGDVLTVTGKTMSENLQGRETSDREVIFPYHEPLAEKAGFLVLKGNLFDFAIMKSSVIGEEFRKRYLSQPGQEGVFEARAIVFDGSDDYHKRINDPALEIDERCILVIRGAGPIGWPGSAEVVNMQPPDHLLKKGIMSLPTLGDGRQSGTADSPSILNASPESAIGGGLSWLRTGDTIRIDLNTGRCDALVDEATIAARKQDGIPAVPATMTPWQEIYRAHASQLDTGGVLEFAVKYQDLAAKLPRHNH

SEQ ID NO: 45 - DNA, 1329 bp, Caulobacter crescentus CB15
gtggtttgtcggcggcttctagcatggaccgcccgcgcccgtgaggccgaggatttcgcgctggtcagacaacctacttgccgtccccacatgttagcgctaccaagtgccgacgaacgcgcgccgccgacggtgtcggcgcttcagacgctcgagttttggggagacgacgccgtgggcgtgagtgaattcctgccggaagattggaaagccgcgaccctgctggggcgcatcgactttggcgaaggcccgacgccggtgctggtgcgcggcggccgcgtcgaggacgtctcgaagatcgcccccaccgtcgctgacctgatgaacgccttccagcccggcgcggtgatcccgcgcggcgaggacaagggtccgctggaagccctcgacatccgcccagtctgggaagacccggacggcgccgcgccggtcaagctgttggcccccgtcgacctgcaatgcctgaaggccgccggcgtgaccttcgcggtctcgacccttgagcgggtcatcgaggagcgcgcgcgcggcgacgccggcgaggcgctgaagatccgcaccctgctggccgaacgcatgggcggcgacctcaagagcgtcgagccgggctcgcagggcgcccagcgcctgaaggacgccctgatcgccgacggcctgtggtcgcagtatctggaagtggcgatcggcccggacgccgagatcttcaccaagggcccgaccctgtcctcgatgggctggggcgaccaggtcggcgtccgctatgacagccactggaacaatcccgagccggaagtcgtgctgctgtgcgacggttcgggcctgatccgcggcgcggcgctgggcaacgacgtcaatctgcgcgacttcgaaggtcgttcggccctgctgctcagcaaggccaaggacaacaacgccagctgcgccatcggtccgttcttccgcctgttcgacgagaccttcggcctggacgacgtccgttcggccgaggtcgagctgaagatcaccggccgcgacaacttcgtgctcgacggcaagtcgaacatgagcctgatcagccgcgacccggccgtgctggccggacaggcctatggcaagcagcaccagtatccggacggctttgctttgttcctgggcaccatgttcgccccgatccaggaccgcgacacccccggccagggtttcacccacaaggtcggcgaccgcgtgcgtgtctcgacgccgaagctgggcgtgctcgagaacgaagtcaccacctgcgacaaggccaagccgtggacgttcggcatctcggccctgatccgcaacctggccggccgcggcctcctctaa

SEQ ID NO: 46 - protein, 442 aa, Caulobacter crescentus CB15
MVCRRLLAWTARAREAEDFALVRQPTCRPHMLALPSADERAPPTVSALQTLEFWGDDAVGVSEFLPEDWKAATLLGRIDFGEGPTPVLVRGGRVEDVSKIAPTVADLMNAFQPGAVIPRGEDKGPLEALDIRPVWEDPDGAAPVKLLAPVDLQCLKAAGVTFAVSTLERVIEERARGDAGEALKIRTLLAERMGGDLKSVEPGSQGAQRLKDALIADGLWSQYLEVAIGPDAEIFTKGPTLSSMGWGDQVGVRYDSHWNNPEPEVVLLCDGSGLIRGAALGNDVNLRDFEGRSALLLSKAKDNNASCAIGPFFRLFDETFGLDDVRSAEVELKITGRDNFVLDGKSNMSLISRDPAVLAGQAYGKQHQYPDGFALFLGTMFAPIQDRDTPGQGFTHKVGDRVRVSTPKLGVLENEVTTCDKAKPWTFGISALIRNLAGRGLL

SEQ ID NO: 47 - DNA, 578 bp, Corynebacterium glutamicum ATCC13869
aaattcctgtgaattagctgatttagtacttttcggaggtgtctattcttaccaaatcgtcaagttgtgggtagagtcacctgaatattaattgcaccgcacgggtgatatatgcttatttgctcaagtagttcgaggttaagtgtattttaggtgaacaaatttcagcttcgggtagaagactttcgatgcgcttcagagcttctattgggaaatctgacaccacttgattaaatagcctacccccgaattgggggattggtcattttttgctgtgaaggtagttttgatgcatatgacctgcgtttataaagaaatgtaaacgtgatcagatcgatataaaagaaacagtttgtactcaggtttgaagcattttctccgattcgcctggcaaaaatctcaattgtcgcttacagtttttctcaacgacaggctgctaagctgctagttcggtggcctagtgagtggcgtttacttggataaaagtaatcccatgtcgtgatcagccattttgggttgtttccatagcaatccaaaggtttcgtctttcgatacctattcaaggagccttcgcctct